European Patent Specification EP 3 334 763 B1, published August 7, 2024. Title: NOVEL ANTI-PD-1 ANTIBODIES. Applicant: WuXi Biologics (Shanghai) Co. Ltd. Open Monoclonal Technology, Inc. The sequence listing filed with the application follows.

SEQUENCE LISTING (68 sequences)

SEQ ID NO: 1 - protein, 7 aa, Homo sapiens
STTYYWV

SEQ ID NO: 2 - DNA, 21 bp, Homo sapiens
agtactacttactactgggtc

SEQ ID NO: 3 - protein, 16 aa, Homo sapiens
SISYSGNTYYNPSLKS

SEQ ID NO: 4 - DNA, 48 bp, Homo sapiens
agtatctcttatagtgggaacacctactacaatccgtccctcaagagt

SEQ ID NO: 5 - protein, 13 aa, Homo sapiens
HLGYNGRYLPFDY

SEQ ID NO: 6 - DNA, 39 bp, Homo sapiens
catctagggtataatgggaggtacctcccctttgactac

SEQ ID NO: 7 - protein, 14 aa, Homo sapiens
TGTSSDVGFYNYVS

SEQ ID NO: 8 - DNA, 42 bp, Homo sapiens
actggaaccagcagtgacgttggtttttataactatgtctcc

SEQ ID NO: 9 - protein, 7 aa, Homo sapiens
DVTNRPS

SEQ ID NO: 10 - DNA, 21 bp, Homo sapiens
gatgtcactaatcggccctca

SEQ ID NO: 11 - protein, 10 aa, Homo sapiens
SSYTSISTWV

SEQ ID NO: 12 - DNA, 30 bp, Homo sapiens
agctcatatacaagcatcagcacttgggtg

SEQ ID NO: 13 - protein, 7 aa, Homo sapiens
SSTYYWG

SEQ ID NO: 14 - DNA, 21 bp, Homo sapiens
agtagtacttactactggggc

SEQ ID NO: 15 - protein, 16 aa, Homo sapiens
SISYSGSTYYNPSLKS

SEQ ID NO: 16 - DNA, 48 bp, Homo sapiens
agtatctcttatagtgggagcacctactacaatccgtccctcaagagt

SEQ ID NO: 17 - protein, 7 aa, Homo sapiens
DVSNRPS

SEQ ID NO: 18 - DNA, 21 bp, Homo sapiens
gatgtcagtaatcggccctca

SEQ ID NO: 19 - protein, 10 aa, Homo sapiens
SSYTNISTWV

SEQ ID NO: 20 - DNA, 30 bp, Homo sapiens
agctcatatacaaacatcagcacttgggtg

SEQ ID NO: 21 - protein, 7 aa, Homo sapiens
STTYYWG

SEQ ID NO: 22 - DNA, 21 bp, Homo sapiens
agtactacttactactggggc

SEQ ID NO: 23 - protein, 16 aa, Homo sapiens
SISYSGTTYYNPSLKS

SEQ ID NO: 24 - DNA, 48 bp, Homo sapiens
agtatctcttatagtgggaccacctactacaacccgtccctcaagagt

SEQ ID NO: 25 - protein, 13 aa, Homo sapiens
HLGYNSNWYPFDY

SEQ ID NO: 26 - DNA, 39 bp, Homo sapiens
catctcgggtataacagcaactggtacccttttgactac

SEQ ID NO: 27 - protein, 14 aa, Homo sapiens
TGTSSDVGSYNRVS

SEQ ID NO: 28 - DNA, 42 bp, Homo sapiens
actggaaccagcagtgacgttggtagttataaccgtgtctcc

SEQ ID NO: 29 - protein, 7 aa, Homo sapiens
EVSNRPS

SEQ ID NO: 30 - DNA, 21 bp, Homo sapiens
gaggtcagtaatcggccctca

SEQ ID NO: 31 - protein, 10 aa, Homo sapiens
SSYTSSSTWV

SEQ ID NO: 32 - DNA, 30 bp, Homo sapiens
agctcatatacaagcagcagcacttgggtg

SEQ ID NO: 33 - protein, 5 aa, Homo sapiens
SHAMS

SEQ ID NO: 34 - DNA, 15 bp, Homo sapiens
agccatgccatgagc

SEQ ID NO: 35 - protein, 17 aa, Homo sapiens
TITGGGGSIYYADSVKG

SEQ ID NO: 36 - DNA, 51 bp, Homo sapiens
actattactggtggtggtggtagcatatactacgcagactccgtgaagggc

SEQ ID NO: 37 - protein, 10 aa, Homo sapiens
NRAGEGYFDY

SEQ ID NO: 38 - DNA, 30 bp, Homo sapiens
aaccgcgctggggagggttactttgactac

SEQ ID NO: 39 - protein, 11 aa, Homo sapiens
GGDNIGNKDVH

SEQ ID NO: 40 - DNA, 33 bp, Homo sapiens
gggggagacaacattggaaataaagatgtgcac

SEQ ID NO: 41 - protein, 7 aa, Homo sapiens
RDSNRPS

SEQ ID NO: 42 - DNA, 21 bp, Homo sapiens
agggatagcaaccggccctct

SEQ ID NO: 43 - protein, 8 aa, Homo sapiens
QVWDSIWV

SEQ ID NO: 44 - DNA, 24 bp, Homo sapiens
caggtgtgggacagcatttgggtg

SEQ ID NO: 45 - protein, 123 aa, Homo sapiens
QLQLQESGPGLVKPSETLTLTCTVSGDSISSTTYYWVWIRQPPGKGLEWIGSISYSGNTYYNPSLKSRVTISVDTSKNHFSLKLSSVAATDTALYYCARHLGYNGRYLPFDYWGQGTLVTVSS

SEQ ID NO: 46 - DNA, 369 bp, Homo sapiens
cagctgcagctgcaggagtcgggcccaggactggtgaagccttcggagaccctgaccctcacctgcactgtctctggtgactccatcagcagtactacttactactgggtctggatccgccagcccccagggaagggactggagtggattgggagtatctcttatagtgggaacacctactacaatccgtccctcaagagtcgagtcaccatatccgtagacacgtccaagaaccacttctccctgaagctgagttctgtggccgccacagacacggctctatattactgtgcgagacatctagggtataatgggaggtacctcccctttgactactggggccagggaaccctggtcaccgtctcctcc

SEQ ID NO: 47 - protein, 110 aa, Homo sapiens
QSALTQPASVSGSPGQSITISCTGTSSDVGFYNYVSWYQQHPGKAPELMIYDVTNRPSGVSDRFSGSKSGNTASLTISGLQAEDEADYYCSSYTSISTWVFGGGTKLTVL

SEQ ID NO: 48 - DNA, 330 bp, Homo sapiens
cagtctgccctgactcagcctgcctccgtgtctgggtctcctggacagtcgatcaccatctcctgcactggaaccagcagtgacgttggtttttataactatgtctcctggtaccaacagcacccaggcaaagcccccgaactcatgatttatgatgtcactaatcggccctcaggggtttctgatcgcttctctggctccaagtctggcaacacggcctccctgaccatctctgggctccaggctgaggacgaggctgattattactgcagctcatatacaagcatcagcacttgggtgttcggcggagggaccaagctgaccgtccta

SEQ ID NO: 49 - protein, 123 aa, Homo sapiens
QLQLQESGPGLVKPSETLSLTCTVSGGSISSSTYYWGWIRQPPGKGLEWIGSISYSGSTYYNPSLKSRVTISVDTSKNQFSLKLSSVTDADTAVYYCARHLGYNGRYLPFDYWGQGTLVTVSS

SEQ ID NO: 50 - DNA, 369 bp, Homo sapiens
cagctgcagctgcaggagtcgggcccaggactggtgaagccttcggagaccctgtccctcacctgcactgtctctggtggctccatcagcagtagtacttactactggggctggatccgccagcccccagggaagggactggagtggattgggagtatctcttatagtgggagcacctactacaatccgtccctcaagagtcgagtcaccatatccgtagacacgtccaagaaccagttctccctgaagctgagctctgtgaccgacgcagacacggctgtgtattactgtgcgagacatctagggtataatgggaggtacctcccctttgactactggggccagggaaccctggtcaccgtctcctcc

SEQ ID NO: 51 - protein, 110 aa, Homo sapiens
QSALTQPASVSGSPGQSITISCTGTSSDVGFYNYVSWYQQHPGKAPEVMIYDVSNRPSGVSDRFSGSKSGNTASLTISGLQAEDEADYYCSSYTSISTWVFGGGTKLTVL

SEQ ID NO: 52 - DNA, 330 bp, Homo sapiens
cagtctgccctgactcagcctgcctccgtgtctgggtctcctggacagtcgatcaccatctcctgcactggaaccagcagtgacgttggtttttataactatgtctcctggtaccaacagcacccaggcaaagcccccgaagtcatgatttatgatgtcagtaatcggccctcaggggtttctgatcgcttctctggctccaagtctggcaacacggcctccctgactatctctgggctccaggctgaggacgaggctgattattactgcagctcatatacaagcatcagcacttgggtgttcggcggagggaccaagctgactgtccta

SEQ ID NO: 53 - protein, 123 aa, Homo sapiens
QLQLQESGPGLVKPSETLTLTCTVSADSISSTTYYWVWIRQPPGKGLEWIGSISYSGSTYYNPSLKSRVTVSVDTSKNQFSLKLNSVAATDTALYYCARHLGYNGRYLPFDYWGQGTLVTVSS

SEQ ID NO: 54 - DNA, 369 bp, Homo sapiens
cagctgcagctgcaggagtcgggcccaggactggtgaagccttcggagaccctgaccctcacctgcactgtctctgctgactccatcagcagtactacttactactgggtctggatccgccagcccccagggaagggactggagtggattgggagtatctcttatagtgggagcacctactacaatccgtccctcaagagtcgagtcaccgtatccgtagacacgtccaagaaccagttctccctgaagctgaactctgtggccgccacagacacggctctatattactgtgcgagacatctagggtataatgggaggtacctcccctttgactactggggccagggaaccctggtcaccgtctcctcc

SEQ ID NO: 55 - protein, 110 aa, Homo sapiens
QSALTQPASVSGSPGQSITISCTGTSSDVGFYNYVSWYQQHPGKAPELMIYDVSNRPSGVSDRFSGSKSGNTASLTISGLQAEDEADYYCSSYTNISTWVFGGGTKLTVL

SEQ ID NO: 56 - DNA, 330 bp, Homo sapiens
cagtctgccctgactcagcctgcctccgtgtctgggtctcctggacagtcgatcaccatctcctgcactggaaccagcagtgacgttggtttttataactatgtctcctggtaccaacagcacccaggcaaagcccccgaactcatgatttatgatgtcagtaatcggccctcaggggtttctgatcgcttctctggctccaagtctggcaacacggcctccctgaccatctctgggctccaggctgaggacgaggctgattattactgcagctcatatacaaacatcagcacttgggtgttcggcggagggaccaagctgaccgtccta

SEQ ID NO: 57 - protein, 123 aa, Homo sapiens
QLQLQESGPGLVKPSETLSLTCTVSGGSISSTTYYWGWIRQPPGKGLEWIGSISYSGTTYYNPSLKSRVTIPVDTSKNQISLKLSSVTAADTSLYYCARHLGYNSNWYPFDYWGQGTLVTVSS

SEQ ID NO: 58 - DNA, 369 bp, Homo sapiens
cagctgcagctgcaggagtcgggcccaggactggtgaagccctcggagaccctgtccctcacctgcactgtctctggtggctccatcagcagtactacttactactggggctggatccgccagcccccagggaaggggctggagtggattgggagtatctcttatagtgggaccacctactacaacccgtccctcaagagtcgagtcaccatccccgtagacacgtccaagaaccagatctccctgaaactgagctctgtgaccgccgcagacacgtctttgtattattgtgcgagacatctcgggtataacagcaactggtacccttttgactactggggccagggaaccctggtcaccgtctcctca

SEQ ID NO: 59 - protein, 110 aa, Homo sapiens
QSALTQPPSVSGSPGQSVTISCTGTSSDVGSYNRVSWYQQPPGTAPEVIIYEVSNRPSGVPDRFSGSKSGNTASLTISGLQAEDEADYYCSSYTSSSTWVFGGGTKLTVL

SEQ ID NO: 60 - DNA, 330 bp, Homo sapiens
cagtcggccctgactcagcctccctccgtgtccgggtctcctggacagtcagtcaccatctcctgcactggaaccagcagtgacgttggtagttataaccgtgtctcctggtaccagcagcccccaggcacagcccccgaagtcattatttatgaggtcagtaatcggccctcaggggtccctgatcgcttctctgggtccaagtctggcaacacggcctccctgaccatctctgggctccaggctgaggacgaggctgattattactgcagctcatatacaagcagcagcacttgggtgttcggcggagggaccaagctgaccgtccta

SEQ ID NO: 61 - protein, 119 aa, Homo sapiens
EVQLLESGGGLVQPGGSLRLSCAASGFTFSSHAMSWVRQAPGKGLEWVSTITGGGGSIYYADSVKGRFTISRDNSKNTLYLQMNSLRAEDTAVYYCAKNRAGEGYFDYWGQGTLVTVSS

SEQ ID NO: 62 - DNA, 357 bp, Homo sapiens
gaggtgcagctgttggagtctgggggaggcttggtacagcctggggggtccctgagactgtcctgcgcagcctctggattcacctttagcagccatgccatgagctgggtccgccaggctccagggaaggggctggagtgggtctcaactattactggtggtggtggtagcatatactacgcagactccgtgaagggccggttcaccatctccagagacaattccaagaacacgctgtatctgcaaatgaacagcctgagagccgaggacacggccgtatattattgtgcgaaaaaccgcgctggggagggttactttgactactggggccagggaaccctggtcaccgtctcctca

SEQ ID NO: 63 - protein, 105 aa, Homo sapiens
SYELTQPLSVSVALGQTARITCGGDNIGNKDVHWYQQKPGQAPVLVIYRDSNRPSGIPEGFSGSNSGNTATLTISRAQAGDEADYYCQVWDSIWVFGGGTKLTVL

SEQ ID NO: 64 - DNA, 315 bp, Homo sapiens
tcctatgagctgactcagccactctcagtgtcagtggccctgggacagacggccaggattacctgtgggggagacaacattggaaataaagatgtgcactggtaccagcagaagccaggccaggcccctgtgctggtcatctatagggatagcaaccggccctctgggatccctgagggattctctggctccaactcggggaacacggccaccctgaccatcagcagagcccaagccggggatgaggctgactattactgtcaggtgtgggacagcatttgggtgttcggcggagggaccaagctgaccgtccta

SEQ ID NO: 65 - protein, 10 aa, Artificial Sequence
  Synthesis
SSYTSISTWV

SEQ ID NO: 66 - DNA, 30 bp, Artificial Sequence; identical to SEQ ID NO: 12
  Synthesis

SEQ ID NO: 67 - protein, 110 aa, Artificial Sequence
  Synthesis
QSALTQPASVSGSPGQSITISCTGTSSDVGFYNYVSWYQQHPGKAPELMIYDVSNRPSGVSDRFSGSKSGNTASLTISGLQAEDEADYYCSSYTSISTWVFGGGTKLTVL

SEQ ID NO: 68 - DNA, 330 bp, Artificial Sequence
  Synthesis
cagtctgccctgactcagcctgcctccgtgtctgggtctcctggacagtcgatcaccatctcctgcactggaaccagcagtgacgttggtttttataactatgtctcctggtaccaacagcacccaggcaaagcccccgaactcatgatttatgatgtcagtaatcggccctcaggggtttctgatcgcttctctggctccaagtctggcaacacggcctccctgaccatctctgggctccaggctgaggacgaggctgattattactgcagctcatatacaagcatcagcacttgggtgttcggcggagggaccaagctgaccgtccta